European Patent Specification EP 3 368 058 B1, published May 3, 2023. Title: A METHOD OF INDUCING CARDIOMYOCYTES PROLIFERATION AND TREATING HEART DISEASES. Applicant: Yeda Research and Development Co. Ltd. TZAHOR, Eldad BASSAT, Elad. The sequence listing filed with the application follows.

SEQUENCE LISTING (38 sequences)

SEQ ID NO: 1 - protein, 4392 aa, Homo sapiens
MGWRAAGALLLALLLHGRLLAVTHGLRAYDGLSLPEDIETVTASQMRWTHSYLSDDEDMLADSISGDDLGSGDLGSGDFQMVYFRALVNFTRSIEYSPQLEDAGSREFREVSEAVVDTLESEYLKIPGDQVVSVVFIKELDGWVFVELDVGSEGNADGAQIQEMLLRVISSGSVASYVTSPQGFQFRRLGTVPQFPRACTEAEFACHSYNECVALEYRCDRRPDCRDMSDELNCEEPVLGISPTFSLLVETTSLPPRPETTIMRQPPVTHAPQPLLPGSVRPLPCGPQEAACRNGHCIPRDYLCDGQEDCEDGSDELDCGPPPPCEPNEFPCGNGHCALKLWRCDGDFDCEDRTDEANCPTKRPEEVCGPTQFRCVSTNMCIPASFHCDEESDCPDRSDEFGCMPPQVVTPPRESIQASRGQTVTFTCVAIGVPTPIINWRLNWGHIPSHPRVTVTSEGGRGTLIIRDVKESDQGAYTCEAMNARGMVFGIPDGVLELVPQRAGPCPDGHFYLEHSAACLPCFCFGITSVCQSTRRFRDQIRLRFDQPDDFKGVNVTMPAQPGTPPLSSTQLQIDPSLHEFQLVDLSRRFLVHDSFWALPEQFLGNKVDSYGGSLRYNVRYELARGMLEPVQRPDVVLMGAGYRLLSRGHTPTQPGALNQRQVQFSEEHWVHESGRPVQRAELLQVLQSLEAVLIQTVYNTKMASVGLSDIAMDTTVTHATSHGRAHSVEECRCPIGYSGLSCESCDAHFTRVPGGPYLGTCSGCNCNGHASSCDPVYGHCLNCQHNTEGPQCNKCKAGFFGDAMKATATSCRPCPCPYIDASRRFSDTCFLDTDGQATCDACAPGYTGRRCESCAPGYEGNPIQPGGKCRPVNQEIVRCDERGSMGTSGEACRCKNNVVGRLCNECADGSFHLSTRNPDGCLKCFCMGVSRHCTSSSWSRAQLHGASEEPGHFSLTNAASTHTTNEGIFSPTPGELGFSSFHRLLSGPYFWSLPSRFLGDKVTSYGGELRFTVTQRSQPGSTPLHGQPLVVLQGNNIILEHHVAQEPSPGQPSTFIVPFREQAWQRPDGQPATREHLLMALAGIDTLLIRASYAQQPAESRVSGISMDVAVPEETGQDPALEVEQCSCPPGYRGPSCQDCDTGYTRTPSGLYLGTCERCSCHGHSEACEPETGACQGCQHHTEGPRCEQCQPGYYGDAQRGTPQDCQLCPCYGDPAAGQAAHTCFLDTDGHPTCDACSPGHSGRHCERCAPGYYGNPSQGQPCQRDSQVPGPIGCNCDPQGSVSSQCDAAGQCQCKAQVEGLTCSHCRPHHFHLSASNPDGCLPCFCMGITQQCASSAYTRHLISTHFAPGDFQGFALVNPQRNSRLTGEFTVEPVPEGAQLSFGNFAQLGHESFYWQLPETYQGDKVAAYGGKLRYTLSYTAGPQGSPLSDPDVQITGNNIMLVASQPALQGPERRSYEIMFREEFWRRPDGQPATREHLLMALADLDELLIRATFSSVPLAASISAVSLEVAQPGPSNRPRALEVEECRCPPGYIGLSCQDCAPGYTRTGSGLYLGHCELCECNGHSDLCHPETGACSQCQHNAAGEFCELCAPGYYGDATAGTPEDCQPCACPLTNPENMFSRTCESLGAGGYRCTACEPGYTGQYCEQCGPGYVGNPSVQGGQCLPETNQAPLVVEVHPARSIVPQGGSHSLRCQVSGSPPHYFYWSREDGRPVPSGTQQRHQGSELHFPSVQPSDAGVYICTCRNLHQSNTSRAELLVTEAPSKPITVTVEEQRSQSVRPGADVTFICTAKSKSPAYTLVWTRLHNGKLPTRAMDFNGILTIRNVQLSDAGTYVCTGSNMFAMDQGTATLHVQASGTLSAPVVSIHPPQLTVQPGQLAEFRCSATGSPTPTLEWTGGPGGQLPAKAQIHGGILRLPAVEPTDQAQYLCRAHSSAGQQVARAVLHVHGGGGPRVQVSPERTQVHAGRTVRLYCRAAGVPSATITWRKEGGSLPPQARSERTDIATLLIPAITTADAGFYLCVATSPAGTAQARIQVVVLSASDASPPPVKIESSSPSVTEGQTLDLNCVVAGSAHAQVTWYRRGGSLPPHTQVHGSRLRLPQVSPADSGEYVCRVENGSGPKEASITVSVLHGTHSGPSYTPVPGSTRPIRIEPSSSHVAEGQTLDLNCVVPGQAHAQVTWHKRGGSLPARHQTHGSLLRLHQVTPADSGEYVCHVVGTSGPLEASVLVTIEASVIPGPIPPVRIESSSSTVAEGQTLDLSCVVAGQAHAQVTWYKRGGSLPARHQVRGSRLYIFQASPADAGQYVCRASNGMEASITVTVTGTQGANLAYPAGSTQPIRIEPSSSQVAEGQTLDLNCVVPGQSHAQVTWHKRGGSLPVRHQTHGSLLRLYQASPADSGEYVCRVLGSSVPLEASVLVTIEPAGSVPALGVTPTVRIESSSSQVAEGQTLDLNCLVAGQAHAQVTWHKRGGSLPARHQVHGSRLRLLQVTPADSGEYVCRVVGSSGTQEASVLVTIQQRLSGSHSQGVAYPVRIESSSASLANGHTLDLNCLVASQAPHTITWYKRGGSLPSRHQIVGSRLRIPQVTPADSGEYVCHVSNGAGSRETSLIVTIQGSGSSHVPSVSPPIRIESSSPTVVEGQTLDLNCVVARQPQAIITWYKRGGSLPSRHQTHGSHLRLHQMSVADSGEYVCRANNNIDALEASIVISVSPSAGSPSAPGSSMPIRIESSSSHVAEGETLDLNCVVPGQAHAQVTWHKRGGSLPSHHQTRGSRLRLHHVSPADSGEYVCRVMGSSGPLEASVLVTIEASGSSAVHVPAPGGAPPIRIEPSSSRVAEGQTLDLKCVVPGQAHAQVTWHKRGGNLPARHQVHGPLLRLNQVSPADSGEYSCQVTGSSGTLEASVLVTIEPSSPGPIPAPGLAQPIYIEASSSHVTEGQTLDLNCVVPGQAHAQVTWYKRGGSLPARHQTHGSQLRLHLVSPADSGEYVCRAASGPGPEQEASFTVTVPPSEGSSYRLRSPVISIDPPSSTVQQGQDASFKCLIHDGAAPISLEWKTRNQELEDNVHISPNGSIITIVGTRPSNHGTYRCVASNAYGVAQSVVNLSVHGPPTVSVLPEGPVWVKVGKAVTLECVSAGEPRSSARWTRISSTPAKLEQRTYGLMDSHAVLQISSAKPSDAGTYVCLAQNALGTAQKQVEVIVDTGAMAPGAPQVQAEEAELTVEAGHTATLRCSATGSPAPTIHWSKLRSPLPWQHRLEGDTLIIPRVAQQDSGQYICNATSPAGHAEATIILHVESPPYATTVPEHASVQAGETVQLQCLAHGTPPLTFQWSRVGSSLPGRATARNELLHFERAAPEDSGRYRCRVTNKVGSAEAFAQLLVQGPPGSLPATSIPAGSTPTVQVTPQLETKSIGASVEFHCAVPSDRGTQLRWFKEGGQLPPGHSVQDGVLRIQNLDQSCQGTYICQAHGPWGKAQASAQLVIQALPSVLINIRTSVQTVVVGHAVEFECLALGDPKPQVTWSKVGGHLRPGIVQSGGVVRIAHVELADAGQYRCTATNAAGTTQSHVLLLVQALPQISMPQEVRVPAGSAAVFPCIASGYPTPDISWSKLDGSLPPDSRLENNMLMLPSVRPQDAGTYVCTATNRQGKVKAFAHLQVPERVVPYFTQTPYSFLPLPTIKDAYRKFEIKITFRPDSADGMLLYNGQKRVPGSPTNLANRQPDFISFGLVGGRPEFRFDAGSGMATIRHPTPLALGHFHTVTLLRSLTQGSLIVGDLAPVNGTSQGKFQGLDLNEELYLGGYPDYGAIPKAGLSSGFIGCVRELRIQGEEIVFHDLNLTAHGISHCPTCRDRPCQNGGQCHDSESSSYVCVCPAGFTGSRCEHSQALHCHPEACGPDATCVNRPDGRGYTCRCHLGRSGLRCEEGVTVTTPSLSGAGSYLALPALTNTHHELRLDVEFKPLAPDGVLLFSGGKSGPVEDFVSLAMVGGHLEFRYELGSGLAVLRSAEPLALGRWHRVSAERLNKDGSLRVNGGRPVLRSSPGKSQGLNLHTLLYLGGVEPSVPLSPATNMSAHFRGCVGEVSVNGKRLDLTYSFLGSQGIGQCYDSSPCERQPCQHGATCMPAGEYEFQCLCRDGFKGDLCEHEENPCQLREPCLHGGTCQGTRCLCLPGFSGPRCQQGSGHGIAESDWHLEGSGGNDAPGQYGAYFHDDGFLAFPGHVFSRSLPEVPETIELEVRTSTASGLLLWQGVEVGEAGQGKDFISLGLQDGHLVFRYQLGSGEARLVSEDPINDGEWHRVTALREGRRGSIQVDGEELVSGRSPGPNVAVNAKGSVYIGGAPDVATLTGGRFSSGITGCVKNLVLHSARPGAPPPQPLDLQHRAQAGANTRPCPS

SEQ ID NO: 2 - protein, 4391 aa, Homo sapiens
MGWRAAGALLLALLLHGRLLAVTHGLRAYDGLSLPEDIETVTASQMRWTHSYLSDDEDMLADSISGDDLGSGDLGSGDFQMVYFRALVNFTRSIEYSPQLEDAGSREFREVSEAVVDTLESEYLKIPGDQVVSVVFIKELDGWVFVELDVGSEGNADGAQIQEMLLRVISSGSVASYVTSPQGFQFRRLGTVPQFPRACTEAEFACHSYNECVALEYRCDRRPDCRDMSDELNCEEPVLGISPTFSLLVETTSLPPRPETTIMRQPPVTHAPQPLLPGSVRPLPCGPQEAACRNGHCIPRDYLCDGQEDCEDGSDELDCGPPPPCEPNEFPCGNGHCALKLWRCDGDFDCEDRTDEANCPTKRPEEVCGPTQFRCVSTNMCIPASFHCDEESDCPDRSDEFGCMPPQVVTPPRESIQASRGQTVTFTCVAIGVPTPIINWRLNWGHIPSHPRVTVTSEGGRGTLIIRDVKESDQGAYTCEAMNARGMVFGIPDGVLELVPQRGPCPDGHFYLEHSAACLPCFCFGITSVCQSTRRFRDQIRLRFDQPDDFKGVNVTMPAQPGTPPLSSTQLQIDPSLHEFQLVDLSRRFLVHDSFWALPEQFLGNKVDSYGGSLRYNVRYELARGMLEPVQRPDVVLMGAGYRLLSRGHTPTQPGALNQRQVQFSEEHWVHESGRPVQRAELLQVLQSLEAVLIQTVYNTKMASVGLSDIAMDTTVTHATSHGRAHSVEECRCPIGYSGLSCESCDAHFTRVPGGPYLGTCSGCNCNGHASSCDPVYGHCLNCQHNTEGPQCNKCKAGFFGDAMKATATSCRPCPCPYIDASRRFSDTCFLDTDGQATCDACAPGYTGRRCESCAPGYEGNPIQPGGKCRPVNQEIVRCDERGSMGTSGEACRCKNNVVGRLCNECADGSFHLSTRNPDGCLKCFCMGVSRHCTSSSWSRAQLHGASEEPGHFSLTNAASTHTTNEGIFSPTPGELGFSSFHRLLSGPYFWSLPSRFLGDKVTSYGGELRFTVTQRSQPGSTPLHGQPLVVLQGNNIILEHHVAQEPSPGQPSTFIVPFREQAWQRPDGQPATREHLLMALAGIDTLLIRASYAQQPAESRVSGISMDVAVPEETGQDPALEVEQCSCPPGYRGPSCQDCDTGYTRTPSGLYLGTCERCSCHGHSEACEPETGACQGCQHHTEGPRCEQCQPGYYGDAQRGTPQDCQLCPCYGDPAAGQAAHTCFLDTDGHPTCDACSPGHSGRHCERCAPGYYGNPSQGQPCQRDSQVPGPIGCNCDPQGSVSSQCDAAGQCQCKAQVEGLTCSHCRPHHFHLSASNPDGCLPCFCMGITQQCASSAYTRHLISTHFAPGDFQGFALVNPQRNSRLTGEFTVEPVPEGAQLSFGNFAQLGHESFYWQLPETYQGDKVAAYGGKLRYTLSYTAGPQGSPLSDPDVQITGNNIMLVASQPALQGPERRSYEIMFREEFWRRPDGQPATREHLLMALADLDELLIRATFSSVPLAASISAVSLEVAQPGPSNRPRALEVEECRCPPGYIGLSCQDCAPGYTRTGSGLYLGHCELCECNGHSDLCHPETGACSQCQHNAAGEFCELCAPGYYGDATAGTPEDCQPCACPLTNPENMFSRTCESLGAGGYRCTACEPGYTGQYCEQCGPGYVGNPSVQGGQCLPETNQAPLVVEVHPARSIVPQGGSHSLRCQVSGSPPHYFYWSREDGRPVPSGTQQRHQGSELHFPSVQPSDAGVYICTCRNLHQSNTSRAELLVTEAPSKPITVTVEEQRSQSVRPGADVTFICTAKSKSPAYTLVWTRLHNGKLPTRAMDFNGILTIRNVQLSDAGTYVCTGSNMFAMDQGTATLHVQASGTLSAPVVSIHPPQLTVQPGQLAEFRCSATGSPTPTLEWTGGPGGQLPAKAQIHGGILRLPAVEPTDQAQYLCRAHSSAGQQVARAVLHVHGGGGPRVQVSPERTQVHAGRTVRLYCRAAGVPSATITWRKEGGSLPPQARSERTDIATLLIPAITTADAGFYLCVATSPAGTAQARIQVVVLSASDASPPPVKIESSSPSVTEGQTLDLNCVVAGSAHAQVTWYRRGGSLPPHTQVHGSRLRLPQVSPADSGEYVCRVENGSGPKEASITVSVLHGTHSGPSYTPVPGSTRPIRIEPSSSHVAEGQTLDLNCVVPGQAHAQVTWHKRGGSLPARHQTHGSLLRLHQVTPADSGEYVCHVVGTSGPLEASVLVTIEASVIPGPIPPVRIESSSSTVAEGQTLDLSCVVAGQAHAQVTWYKRGGSLPARHQVRGSRLYIFQASPADAGQYVCRASNGMEASITVTVTGTQGANLAYPAGSTQPIRIEPSSSQVAEGQTLDLNCVVPGQSHAQVTWHKRGGSLPVRHQTHGSLLRLYQASPADSGEYVCRVLGSSVPLEASVLVTIEPAGSVPALGVTPTVRIESSSSQVAEGQTLDLNCLVAGQAHAQVTWHKRGGSLPARHQVHGSRLRLLQVTPADSGEYVCRVVGSSGTQEASVLVTIQQRLSGSHSQGVAYPVRIESSSASLANGHTLDLNCLVASQAPHTITWYKRGGSLPSRHQIVGSRLRIPQVTPADSGEYVCHVSNGAGSRETSLIVTIQGSGSSHVPSVSPPIRIESSSPTVVEGQTLDLNCVVARQPQAIITWYKRGGSLPSRHQTHGSHLRLHQMSVADSGEYVCRANNNIDALEASIVISVSPSAGSPSAPGSSMPIRIESSSSHVAEGETLDLNCVVPGQAHAQVTWHKRGGSLPSHHQTRGSRLRLHHVSPADSGEYVCRVMGSSGPLEASVLVTIEASGSSAVHVPAPGGAPPIRIEPSSSRVAEGQTLDLKCVVPGQAHAQVTWHKRGGNLPARHQVHGPLLRLNQVSPADSGEYSCQVTGSSGTLEASVLVTIEPSSPGPIPAPGLAQPIYIEASSSHVTEGQTLDLNCVVPGQAHAQVTWYKRGGSLPARHQTHGSQLRLHLVSPADSGEYVCRAASGPGPEQEASFTVTVPPSEGSSYRLRSPVISIDPPSSTVQQGQDASFKCLIHDGAAPISLEWKTRNQELEDNVHISPNGSIITIVGTRPSNHGTYRCVASNAYGVAQSVVNLSVHGPPTVSVLPEGPVWVKVGKAVTLECVSAGEPRSSARWTRISSTPAKLEQRTYGLMDSHAVLQISSAKPSDAGTYVCLAQNALGTAQKQVEVIVDTGAMAPGAPQVQAEEAELTVEAGHTATLRCSATGSPAPTIHWSKLRSPLPWQHRLEGDTLIIPRVAQQDSGQYICNATSPAGHAEATIILHVESPPYATTVPEHASVQAGETVQLQCLAHGTPPLTFQWSRVGSSLPGRATARNELLHFERAAPEDSGRYRCRVTNKVGSAEAFAQLLVQGPPGSLPATSIPAGSTPTVQVTPQLETKSIGASVEFHCAVPSDRGTQLRWFKEGGQLPPGHSVQDGVLRIQNLDQSCQGTYICQAHGPWGKAQASAQLVIQALPSVLINIRTSVQTVVVGHAVEFECLALGDPKPQVTWSKVGGHLRPGIVQSGGVVRIAHVELADAGQYRCTATNAAGTTQSHVLLLVQALPQISMPQEVRVPAGSAAVFPCIASGYPTPDISWSKLDGSLPPDSRLENNMLMLPSVRPQDAGTYVCTATNRQGKVKAFAHLQVPERVVPYFTQTPYSFLPLPTIKDAYRKFEIKITFRPDSADGMLLYNGQKRVPGSPTNLANRQPDFISFGLVGGRPEFRFDAGSGMATIRHPTPLALGHFHTVTLLRSLTQGSLIVGDLAPVNGTSQGKFQGLDLNEELYLGGYPDYGAIPKAGLSSGFIGCVRELRIQGEEIVFHDLNLTAHGISHCPTCRDRPCQNGGQCHDSESSSYVCVCPAGFTGSRCEHSQALHCHPEACGPDATCVNRPDGRGYTCRCHLGRSGLRCEEGVTVTTPSLSGAGSYLALPALTNTHHELRLDVEFKPLAPDGVLLFSGGKSGPVEDFVSLAMVGGHLEFRYELGSGLAVLRSAEPLALGRWHRVSAERLNKDGSLRVNGGRPVLRSSPGKSQGLNLHTLLYLGGVEPSVPLSPATNMSAHFRGCVGEVSVNGKRLDLTYSFLGSQGIGQCYDSSPCERQPCQHGATCMPAGEYEFQCLCRDGFKGDLCEHEENPCQLREPCLHGGTCQGTRCLCLPGFSGPRCQQGSGHGIAESDWHLEGSGGNDAPGQYGAYFHDDGFLAFPGHVFSRSLPEVPETIELEVRTSTASGLLLWQGVEVGEAGQGKDFISLGLQDGHLVFRYQLGSGEARLVSEDPINDGEWHRVTALREGRRGSIQVDGEELVSGRSPGPNVAVNAKGSVYIGGAPDVATLTGGRFSSGITGCVKNLVLHSARPGAPPPQPLDLQHRAQAGANTRPCPS

SEQ ID NO: 3 - protein, 4383 aa, Mus musculus
MGQRAVGSLLLGLLLHARLLAVTHGLRAYDGLSLPEDTETVTASRYGWTYSYLSDDEDLLADDASGDGLGSGDVGSGDFQMVYFRALVNFTRSIEYSPQLEDASAKEFREVSEAVVEKLEPEYRKIPGDQIVSVVFIKELDGWVFVELDVGSEGNADGSQIQEVLHTVVSSGSIGPYVTSPWGFKFRRLGTVPQFPRVCTETEFACHSYNECVALEYRCDRRPDCRDMSDELNCEEPVPELSSSTPAVGKVSPLPLWPEAATTPPPPVTHGPQFLLPSVPGPSACGPQEASCHSGHCIPRDYLCDGQEDCRDGSDELGCASPPPCEPNEFACENGHCALKLWRCDGDFDCEDRTDEANCSVKQPGEVCGPTHFQCVSTNRCIPASFHCDEESDCPDRSDEFGCMPPQVVTPPQQSIQASRGQTVTFTCVATGVPTPIINWRLNWGHIPAHPRVTMTSEGGRGTLIIRDVKEADQGAYTCEAMNSRGMVFGIPDGVLELVPQRGPCPDGHFYLEDSASCLPCFCFGVTNVCQSSLRFRDQIRLSFDQPNDFKGVNVTMPSQPGVPPLSSTQLQIDPALQEFQLVDLSRRFLVHDAFWALPKQFLGNKVDSYGGFLRYKVRYELARGMLEPVQKPDVILVGAGYRLHSRGHTPTHPGTLNQRQVQLSEEHWVHESGRPVQRAEMLQALASLEAVLLQTVYNTKMASVGLSDIVMDTTVTHTTIHGRAHSVEECRCPIGYSGLSCESCDAHFTRVPGGPYLGTCSGCNCNGHASSCDPVYGHCLNCQHNTEGPQCDKCKPGFFGDATKATATACRPCPCPYIDASRRFSDTCFLDTDGQATCDACAPGYTGRRCESCAPGYEGNPIQPGGKCRPTTQEIVRCDERGSLGTSGETCRCKNNVVGRLCNECSDGSFHLSKQNPDGCLKCFCMGVSRQCSSSSWSRAQVLGASEQPSQFSLSNAAGTHTTSEGVSSPAPGELSFSSFHNLLSEPYFWSLPASFRGDKVTSYGGELRFTVTQRPRPSSAPLHRQPLVVLQGNNIVLEHHASRDPSPGQPSNFIVPFQEQAWQRPDGQPATREHLLMALAGIDALLIQASYTQQPAESRVSGISMDVAVPENTGQDSAREVEQCTCPPGYRGPSCQDCDTGYTRVPSGLYLGTCERCNCHGHSETCEPETGACQSCQHHTEGASCEQCQPGYYGDAQRGTPQDCQPCPCYGAPAAGQAAHTCFLDTDGHPTCDSCSPGHSGRHCERCAPGYYGNPSQGQPCHRDGQVPEVLGCGCDPHGSISSQCDAAGQCQCKAQVEGRTCSHCRPHHFHLSASNPEGCLPCFCMGVTQQCASSSYSRQLISTHFAPGDFQGFALVNPQRNSQLTGGFTVEPVHDGARLSFSNFAHLGQESFYWQLPEIYQGDKVAAYGGKLRYTLSYTAGPQGSPLLDPDIQITGNNIMLVASQPALQGPERRSYEIIFREEFWRRPDGQPATREHLLMALADLDELLVRATFSSVPRAASISAVSLEVAQPGPSSGPRALEVEECRCPPGYVGLSCQDCAPGYTRTGSGLYLGQCELCECNGHSDLCHPETGACSRCQHNTAGEFCELCATGYYGDATAGTPEDCQPCACPLTNPENMFSRTCESLGAGGYRCTACEPGYTGQYCEQCAPGYEGDPNVQGGRCQPLTKESLEVQIHPSRSVVPQGGPHSLRCQVSGSPPHYFYWSREDGRPLPSSAQQRHQGSELHFPSVQPSDAGVYICTCRNLIHTSNSRAELLVAEAPSKPITVTVEEQRSQSVRPGADVTFICTAKSKSPAYTLVWTRLHNGKLPSRAMDFNGILTIRNVQPSDAGTYVCTGSNMFAMDQGTATLHVQVSGTSTAPVASIHPPQLTVQPGQQAEFRCSATGNPTPMLEWIGGPSGQLPAKAQIHNGILRLPAIEPSDQGQYLCRALSSAGQHVARAMLQVHGGSGPRVQVSPERTQVHEGRTVRLYCRAAGVPSASITWRKEGGSLPPQARSENTDIPTLLIPAITAADAGFYLCVATSPTGTAQARIQVVVLSASGANSVPVRIESSSPSVTEGQTLDLNCAVMGLTYTQVTWYKRGGSLPPHAQVHGSRLRLPQVSPADSGDYVCRVESDVGPKEASIVVSVLHSPHSGPSYTPATSITPPIRIESSSSHVAEGQTLDLNCVVPGQAQVTWRKRGGSLPARHQTHGSLLRLHQVSPADSGEYVCHVVLGSEHTETSVLVTIEPAESIPAPGPAPPVRIEASSSTVTEGHMLDLNCVVAGQAHAQVTWYKRGGSLPARHQVRGSRLYILQASPADAGEYVCRAGNGQEATITVTVTRNHGANLAYPPGSTSPIRIESSSSHVAEGQTLDLNCVVQGQAHAQVTWHKRGGSLPARHQTHGSLLRLHQVSPVDSGEYVCRVEGGAVPLESSVLVTIEPAGTAPGVIPPVRIESSSSHVSEGQSLDLNCLVSGQTHPQISWHKRGGSLPARHQVHGSRLRLLQVTPTDSGEYVCRVVSGSGTQEASILVTIQQTLSPSHSQSVVHPVRIESSSPSLANGHTLDLNCLVASLTPHTITWYKRGGSLPSRHQIVGSRLRIPQVTPADSGEYVCHVSNGAGSQETSLIVTIESRGPSHVPSVSPPMRIETSSPTVTEGQTLDLNCVVVGRPQATITWYKRGGSLPFRHQAHGSRLRLHHMSVADSGEYVCRANNNIDAQETSIMISVSPSTNSPPAPASPAPIRIESSSSRVAEGQTLDLNCVVPGHAHAQVTWHKRGGSLPTHHQTHGSRLRLYQVSSADSGEYVCSVLSSSGPLEASVLVSITPAAANVHIPGEVPFPPIRIETSSSRVAEGQTLDLSCVVPGQAHAQVTWHKRGGSLPAGHQVHGHMLRLNRVSPADSGEYSCQVTGSSGTLEASVLVTIEASEPSPIPAPGLAQPVYIESSSSHLTEGQTVDLKCVVPGQAHAQVTWHKRGSSLPARHQTHGSLLRLYQLSPADSGEYVCQVAGSSHPEHEASFKLTVPSSQNSSFRLRSPVISIEPPSSTVQQGQDASFKCLIHEGATPIKVEWKIRDQELEDNVHISPNGSIITIVGTRPSNHGAYRCVASNVYGMAQSVVNLSVHGPPTVSVLPEGPVHVKMGKDITLECISSGEPRSSPRWTRLGIPVKLEPRMFGLMNSHAMLKIASVKPSDAGTYVCQAQNALGTAQKQVELIVDTGTVAPGAPQVQVEESELTLEAGHTATLHCSATGNPPPTIHWSKLRAPLPWQHRIEGNTLVIPRVAQQDSGQYICNATNSAGHTEATVVLHVESPPYATIIPEHTSAQPGNLVQLQCLAHGTPPLTYQWSLVGGVLPEKAVARNQVLRLEPTVPEDSGRYRCQVSNRVGSAEAFAQVLVQGSSSNLPDTSIPGGSTPTVQVTPQLETRNIGASVEFHCAVPNERGTHLRWLKEGGQLPPGHSVQDGVLRIQNLDQSCQGTYVCQAHGPWGQAQATAQLIVQALPSVLINVRTSVHSVVVGHSVEFECLALGDPKPQVTWSKVGGHLRPGIVQSGSIIRIAHVELADAGQYRCAATNAAGTTQSHVLLLVQALPQISTPPEIRVPAGSAAVFPCMASGYPTPAITWSKVDGDLPPDSRLENNMLMLPSVRPEDAGTYVCTATNRQGKVKAFAYLQVPERVIPYFTQTPYSFLPLPTIKDAYRKFEIKITFRPDSADGMLLYNGQKRSPTNLANRQPDFISFGLVGGRPEFRFDAGSGMATIRHPTPLALGQFHTVTLLRSLTQGSLIVGNLAPVNGTSQGKFQGLDLNEELYLGGYPDYGAIPKAGLSSGFVGCVRELRIQGEEVVFHDVNLTTHGISHCPTCQDRPCQNGGQCQDSESSSYTCVCPAGFTGSRCEHSQALHCHPEACGPDATCVNRPDGRGYTCRCHLGRSGVRCEEGVTVTTPSMSGAGSYLALPALTNMHHELRLDVEFKPLEPNGILLFSGGKSGPVEDFVSLAMVGGHLEFRYELGSGLAVLRSHEPLTLGRWHRVSAERLNKDGSLRVDGGRPVLRSSPGKSQGLNLHTLLYLGGVEPSVQLSPATNMSAHFHGCVGEVSVNGKRLDLTYSFLGSQGVGQCYDSSPCERQPCQNGATCMPAGEYEFQCLCQDGFKGDLCEHEENPCQLHEPCLNGGTCRGARCLCLPGFSGPRCQQGAGYGVVESDWHPEGSGGNDAPGQYGAYFYDNGFLGLPGNSFSRSLPEVPETIEFEVRTSTADGLLLWQGVVREASRSKDFISLGLQDGHLVFSYQLGSGEARLVSEDPINDGEWHRITALREGQRGSIQVDGEDLVTGRSPGPNVAVNTKDIIYIGGAPDVATLTRGKFSSGITGCIKNLVLHTARPGAPPPQPLDLQHRAQAGANTRPCPS

SEQ ID NO: 4 - protein, 2068 aa, Homo sapiens
MAGRSHPGPLRPLLPLLVVAACVLPGAGGTCPERALERREEEANVVLTGTVEEILNVDPVQHTYSCKVRVWRYLKGKDLVARESLLDGGNKVVISGFGDPLICDNQVSTGDTRIFFVNPAPPYLWPAHKNELMLNSSLMRITLRNLEEVEFCVEDKPGTHFTPVPPTPPDACRGMLCGFGAVCEPNAEGPGRASCVCKKSPCPSVVAPVCGSDASTYSNECELQRAQCSQQRRIRLLSRGPCGSRDPCSNVTCSFGSTCARSADGLTASCLCPATCRGAPEGTVCGSDGADYPGECQLLRRACARQENVFKKFDGPCDPCQGALPDPSRSCRVNPRTRRPEMLLRPESCPARQAPVCGDDGVTYENDCVMGRSGAARGLLLQKVRSGQCQGRDQCPEPCRFNAVCLSRRGRPRCSCDRVTCDGAYRPVCAQDGRTYDSDCWRQQAECRQQRAIPSKHQGPCDQAPSPCLGVQCAFGATCAVKNGQAACECLQACSSLYDPVCGSDGVTYGSACELEATACTLGREIQVARKGPCDRCGQCRFGALCEAETGRCVCPSECVALAQPVCGSDGHTYPSECMLHVHACTHQISLHVASAGPCETCGDAVCAFGAVCSAGQCVCPRCEHPPPGPVCGSDGVTYGSACELREAACLQQTQIEEARAGPCEQAECGSGGSGSGEDGDCEQELCRQRGGIWDEDSEDGPCVCDFSCQSVPGSPVCGSDGVTYSTECELKKARCESQRGLYVAAQGACRGPTFAPLPPVAPLHCAQTPYGCCQDNITAARGVGLAGCPSACQCNPHGSYGGTCDPATGQCSCRPGVGGLRCDRCEPGFWNFRGIVTDGRSGCTPCSCDPQGAVRDDCEQMTGLCSCKPGVAGPKCGQCPDGRALGPAGCEADASAPATCAEMRCEFGARCVEESGSAHCVCPMLTCPEANATKVCGSDGVTYGNECQLKTIACRQGLQISIQSLGPCQEAVAPSTHPTSASVTVTTPGLLLSQALPAPPGALPLAPSSTAHSQTTPPPSSRPRTTASVPRTTVWPVLTVPPTAPSPAPSLVASAFGESGSTDGSSDEELSGDQEASGGGSGGLEPLEGSSVATPGPPVERASCYNSALGCCSDGKTPSLDAEGSNCPATKVFQGVLELEGVEGQELFYTPEMADPKSELFGETARSIESTLDDLFRNSDVKKDFRSVRLRDLGPGKSVRAIVDVHFDPTTAFRAPDVARALLRQIQVSRRRSLGVRRPLQEHVRFMDFDWFPAFITGATSGAIAAGATARATTASRLPSSAVTPRAPHPSHTSQPVAKTTAAPTTRRPPTTAPSRVPGRRPPAPQQPPKPCDSQPCFHGGTCQDWALGGGFTCSCPAGRGGAVCEKVLGAPVPAFEGRSFLAFPTLRAYHTLRLALEFRALEPQGLLLYNGNARGKDFLALALLDGRVQLRFDTGSGPAVLTSAVPVEPGQWHRLELSRHWRRGTLSVDGETPVLGESPSGTDGLNLDTDLFVGGVPEDQAAVALERTFVGAGLRGCIRLLDVNNQRLELGIGPGAATRGSGVGECGDHPCLPNPCHGGAPCQNLEAGRFHCQCPPGRVGPTCADEKSPCQPNPCHGAAPCRVLPEGGAQCECPLGREGTFCQTASGQDGSGPFLADFNGFSHLELRGLHTFARDLGEKMALEVVFLARGPSGLLLYNGQKTDGKGDFVSLALRDRRLEFRYDLGKGAAVIRSREPVTLGAWTRVSLERNGRKGALRVGDGPRVLGESPKSRKVPHTVLNLKEPLYVGGAPDFSKLARAAAVSSGFDGAIQLVSLGGRQLLTPEHVLRQVDVTSFAGHPCTRASGHPCLNGASCVPREAAYVCLCPGGFSGPHCEKGLVEKSAGDVDTLAFDGRTFVEYLNAVTESELANEIPVPETLDSGALHSEKALQSNHFELSLRTEATQGLVLWSGKATERADYVALAIVDGHLQLSYNLGSQPVVLRSTVPVNTNRWLRVVAHREQREGSLQVGNEAPVTGSSPLGATQLDTDGALWLGGLPELPVGPALPKAYGTGFVGCLRDVVVGRHPLHLLEDAVTKPELRPCPTP

SEQ ID NO: 5 - protein, 2045 aa, Homo sapiens
MAGRSHPGPLRPLLPLLVVAACVLPGAGGTCPERALERREEEANVVLTGTVEEILNVDPVQHTYSCKVRVWRYLKGKDLVARESLLDGGNKVVISGFGDPLICDNQVSTGDTRIFFVNPAPPYLWPAHKNELMLNSSLMRITLRNLEEVEFCVEDKPGTHFTPVPPTPPDACRGMLCGFGAVCEPNAEGPGRASCVCKKSPCPSVVAPVCGSDASTYSNECELQRAQCSQQRRIRLLSRGPCGSRDPCSNVTCSFGSTCARSADGLTASCLCPATCRGAPEGTVCGSDGADYPGECQLLRRACARQENVFKKFDGPCDPCQGALPDPSRSCRVNPRTRRPEMLLRPESCPARQAPVCGDDGVTYENDCVMGRSGAARGLLLQKVRSGQCQGRDQCPEPCRFNAVCLSRRGRPRCSCDRVTCDGAYRPVCAQDGRTYDSDCWRQQAECRQQRAIPSKHQGPCDQAPSPCLGVQCAFGATCAVKNGQAACECLQACSSLYDPVCGSDGVTYGSACELEATACTLGREIQVARKGPCDRCGQCRFGALCEAETGRCVCPSECVALAQPVCGSDGHTYPSECMLHVHACTHQISLHVASAGPCETCGDAVCAFGAVCSAGQCVCPRCEHPPPGPVCGSDGVTYGSACELREAACLQQTQIEEARAGPCEQAECGSGGSGSGEDGDCEQELCRQRGGIWDEDSEDGPCVCDFSCQSVPGSPVCGSDGVTYSTECELKKARCESQRGLYVAAQGACRGPTFAPLPPVAPLHCAQTPYGCCQDNITAARGVGLAGCPSACQCNPHGSYGGTCDPATGQCSCRPGVGGLRCDRCEPGFWNFRGIVTDGRSGCTPCSCDPQGAVRDDCEQMTGLCSCKPGVAGPKCGQCPDGRALGPAGCEADASAPATCAEMRCEFGARCVEESGSAHCVCPMLTCPEANATKVCGSDGVTYGNECQLKTIACRQGLQISIQSLGPCQEAVAPSTHPTSASVTVTTPGLLLSQALPAPPGALPLAPSSTAHSQTTPPPSSRPRTTASVPRTTVWPVLTVPPTAPSPAPSLVASAFGESGSTDGSSDEELSGDQEASGGGSGGLEPLEGSSVATPGPPVERASCYNSALGCCSDGKTPSLDAEGSNCPATKVFQGVLELEGVEGQELFYTPEMADPKSELFGETARSIESTLDDLFRNSDVKKDFRSVRLRDLGPGKSVRAIVDVHFDPTTAFRAPDVARALLRQIQVSRRRSLGVRRPLQEHVRFMDFDWFPAFITGATSGAIAAGATARATTASRLPSSAVTPRAPHPSHTSQPVAKTTAAPTTRRPPTTAPSRVPGRRPPAPQQPPKPCDSQPCFHGGTCQDWALGGGFTCSCPAGRGGAVCEKVLGAPVPAFEGRSFLAFPTLRAYHTLRLALEFRALEPQGLLLYNGNARGKDFLALALLDGRVQLRFDTGSGPAVLTSAVPVEPGQWHRLELSRHWRRGTLSVDGETPVLGESPSGTDGLNLDTDLFVGGVPEDQAAVALERTFVGAGLRGCIRLLDVNNQRLELGIGPGAATRGSGVGECGDHPCLPNPCHGGAPCQNLEAGRFHCQCPPGRVGPTCADEKSPCQPNPCHGAAPCRVLPEGGAQCECPLGREGTFCQTASGQDGSGPFLADFNGFSHLELRGLHTFARDLGEKMALEVVFLARGPSGLLLYNGQKTDGKGDFVSLALRDRRLEFRYDLGKGAAVIRSREPVTLGAWTRVSLERNGRKGALRVGDGPRVLGESPVPHTVLNLKEPLYVGGAPDFSKLARAAAVSSGFDGAIQLVSLGGRQLLTPEHVLRQVDVTSFAGHPCTRASGHPCLNGASCVPREAAYVCLCPGGFSGPHCEKGLVEKSAGDVDTLAFDGRTFVEYLNAVTESEKALQSNHFELSLRTEATQGLVLWSGKATERADYVALAIVDGHLQLSYNLGSQPVVLRSTVPVNTNRWLRVVAHREQREGSLQVGNEAPVTGSSPLGATQLDTDGALWLGGLPELPVGPALPKAYGTGFVGCLRDVVVGRHPLHLLEDAVTKPELRPCPTP

SEQ ID NO: 6 - protein, 1940 aa, Rattus norvegicus
MPPLPLEHRPRQEPGASMLVRYFMIPCNICLILLATSTLGFAVLLFLSNYKPGIHFTPAPPTPPDVCRGMLCGFGAVCEPSVEDPGRASCVCKKNACPATVAPVCGSDASTYSNECELQRAQCNQQRRIRLLRQGPCGSRDPCANVTCSFGSTCVPSADGQTASCLCPTTCFGAPDGTVCGSDGVDYPSECQLLSHACASQEHIFKKFNGPCDPCQGSMSDLNHICRVNPRTRHPEMLLRPENCPAQHTPICGDDGVTYENDCVMSRIGATRGLLLQKVRSGQCQTRDQCPETCQFNSVCLSRRGRPHCSCDRVTCDGSYRPVCAQDGHTYNNDCWRQQAECRQQRAIPPKHQGPCDQTPSPCHGVQCAFGAVCTVKNGKAECECQRVCSGIYDPVCGSDGVTYGSVCELESMACTLGREIQVARRGPCDPCGQCRFGSLCEVETGRCVCPSECVESAQPVCGSDGHTYASECELHVHACTHQISLYVASAGHCQTCGEKVCTFGAVCSAGQCVCPRCEHPPPGPVCGSDGVTYLSACELREAACQQQVQIEEAHAGPCEPAECGSGGSGSGEDDECEQELCRQRGGIWDEDSEDGPCVCDFSCQSVPRSPVCGSDGVTYGTECDLKKARCESQQELYVAAQGACRGPTLAPLLPVAFPHCAQTPYGCCQDNFTAAQGVGLAGCPSTCHCNPHGSYSGTCDPATGQCSCRPGVGGLRCDRCEPGFWNFRGIVTDGHSGCTPCSCDPRGAVRDDCEQMTGLCSCRPGVAGPKCGQCPDGQVLGHLGCEADPMTPVTCVEIHCEFGASCVEKAGFAQCICPTLTCPEANSTKVCGSDGVTYGNECQLKAIACRQRLDISTQSLGPCQESVTPGASPTSASMTTPRHILSKTLPFPHNSLPLSPGSTTHDWPTPLPISPHTTVSIPRSTAWPVLTVPPTAAASDVTSLATSIFSESGSANGSGDEELSGDEEASGGGSGGLEPPVGSIVVTHGPPIERASCYNSPLGCCSDGKTPSLDSEGSNCPATKAFQGVLELEGVEGQELFYTPEMADPKSELFGETARSIESTLDDLFRNSDVKKDFWSVRLRELGPGKLVRAIVDVHFDPTTAFQASDVGQALLRQIQVSRPWALAVRRPLQEHVRFLDFDWFPTFFTGAATGTTAAMATARATTVSRLPASSVTPRVYPSHTSRPVGRTTAPPTTRRPPTTATNMDRPRTPGHQQPSKSCDSQPCLHGGTCQDQDSGKGFTCSCTAGRGGSVCEKVQPPSMPAFKGHSFLAFPTLRAYHTLRLALEFRALETEGLLLYNGNARGKDFLALALLDGRVQFRFDTGSGPAVLTSLVPVEPGRWHRLELSRHWRQGTLSVDGETPVVGESPSGTDGLNLDTNLYVGGIPEEQVAMVLDRTSVGVGLKGCIRMLDINNQQLELSDWQRAAVQSSGVGECGDHPCLPNPCHGGALCQALEAGMFLCQCPPGRFGPTCADEKSPCQPNPCHGAAPCRVLSSGGAKCECPLGRSGTFCQTVLETAGSRPFLADFNGFSYLELKGLHTFERDLGEKMALEMVFLARGPSGLLLYNGQKTDGKGDFVSLALHNRHLEFCYDLGKGAAVIRSKEPIALGTWVRVFLERNGRKGALQVGDGPRVLGESPKSRKVPHTMLNLKEPLYIGGAPDFSKLARGAAVSSGFSGVIQLVSLRGHQLLTQEHVLRAVDVSPFADHPCTQALGNPCLNGGSCVPREATYECLCPGGFSGLHCEKGLVEKSVGDLETLAFDGRTYIEYLNAVIESEKALQSNHFELSLRTEATQGLVLWIGKAAERADYMALAIVDGHLQLSYDLGSQPVVLRSTVKVNTNRWLRIRAHREHREGSLQVGNEAPVTGSSPLGATQLDTDGALWLGGLQKLPVGQALPKAYGTGFVGCLRDVVVGHRQLHLLEDAVTKPELRPCPTP

SEQ ID NO: 7 - protein, 452 aa, Artificial Sequence
  Amino acid sequence encoding Minimal human  Agrin human sequence - G1 + G2
GAPVPAFEGRSFLAFPTLRAYHTLRLALEFRALEPQGLLLYNGNARGKDFLALALLDGRVQLRFDTGSGPAVLTSAVPVEPGQWHRLELSRHWRRGTLSVDGETPVLGESPSGTDGLNLDTDLFVGGVPEDQAAVALERTFVGAGLRGCIRLLDVNNQRLELGIGPGAATRGSGVGECGDHPCLPNPCHGGAPCQNLEAGRFHCQCPPGRVGPTCADEKSPCQPNPCHGAAPCRVLPEGGAQCECPLGREGTFCQTASGQDGSGPFLADFNGFSHLELRGLHTFARDLGEKMALEVVFLARGPSGLLLYNGQKTDGKGDFVSLALRDRRLEFRYDLGKGAAVIRSREPVTLGAWTRVSLERNGRKGALRVGDGPRVLGESPKSRKVPHTVLNLKEPLYVGGAPDFSKLARAAAVSSGFDGAIQLVSLGGRQLLTPEHVLRQVDVTSFAGHPC

SEQ ID NO: 8 - protein, 188 aa, Artificial Sequence
  Amino acid sequence encoding Minimal human  Agrin human sequence -  G2 only
PFLADFNGFSHLELRGLHTFARDLGEKMALEVVFLARGPSGLLLYNGQKTDGKGDFVSLALRDRRLEFRYDLGKGAAVIRSREPVTLGAWTRVSLERNGRKGALRVGDGPRVLGESPKSRKVPHTVLNLKEPLYVGGAPDFSKLARAAAVSSGFDGAIQLVSLGGRQLLTPEHVLRQVDVTSFAGHPC

SEQ ID NO: 9 - protein, 2034 aa, Mus musculus
MVRPRLSFPAPLLPLLLLLAAAAPAVPGASGTCPERALERREEEANVVLTGTVEEILNVDPVQHTYSCKVRVWRYLKGKDVVAQESLLDGGNKVVIGGFGDPLICDNQVSTGDTRIFFVNPAPPYLWPAHKNELMLNSSLMRITLRNLEEVEFCVEDKPGIHFTAAPSMPPDVCRGMLCGFGAVCEPSVEDPGRASCVCKKNVCPAMVAPVCGSDASTYSNECELQRAQCNQQRRIRLLRQGPCGSRDPCANVTCSFGSTCVPSADGQTASCLCPTTCFGAPDGTVCGSDGVDYPSECQLLRHACANQEHIFKKFDGPCDPCQGSMSDLNHICRVNPRTRHPEMLLRPENCPAQHTPICGDDGVTYENDCVMSRIGAARGLLLQKVRSGQCQTRDQCPETCQFNSVCLSRRGRPHCSCDRVTCDGAYRPVCAQDGHTYDNDCWRQQAECRQQQTIPPKHQGPCDQTPSPCRGAQCAFGATCTVKNGKAVCECQRVCSGGYDPVCGSDGVTYGSVCELESMACTLGREIRVARRGPCDRCGQCRFGSLCEVETGRCVCPSECVESAQPVCGSDGHTYASECELHVHACTHQISLYVASAGHCQTCGETVCTFGAVCSAGQCVCPRCEHPPPGPVCGSDGVTYLSACELREAACQQQVQIEEARAGPCEPAECGSGGSGSGEDNACEQELCRQHGGVWDEDSEDGPCVCDFSCQSVLKSPVCGSDGVTYSTECHLKKARCEARQELYVAAQGACRGPTLAPLLPMASPHCAQTPYGCCQDNVTAAQGVGLAGCPSTCHCNPHGSYSGTCDPVTGQCSCRPGVGGLRCDRCEPGFWNFRGIVTDGHSGCTPCSCDPRGAVRDDCEQMTGLCSCRPGVAGPKCGQCPDGQALGHLGCEADPTTPVTCVEMHCEFGASCVEEAGFAQCVCPTLTCPEANSTKVCGSDGVTYGNECQLKTIACRQRLDISIQSLGPCRESVAPGVSPTSASMTTPRHILSRTLASPHSSLPLSPSTTAHDWPTPLPTSPQTVVGTPRSTAATPSDVASLATAIFRESGSTNGSGDEELSGDEEASGGGSGGLEPPVGSVVVTHGPPIERASCYNSPLGCCSDGKTPSLDSEGSNCPATKAFQGVLELEGVEGQELFYTPEMADPKSELFGETARSIESTLDDLFRNSDVKKDFWSIRLRELGPGKLVRAIVDVHFDPTTAFQAPDVGQALLQQIQVSRPWALAVRRPLREHVRFLDFDWFPTFFTGAATGTTAAVATARATTVSRLSASSVTPRVYPSYTSRPVGRTTAPLTTRRPPTTTASIDRPRTPGPQRPPKSCDSQPCLHGGTCQDLDSGKGFSCSCTAGRAGTVCEKVQLPSVPAFKGHSFLAFPTLRAYHTLRLALEFRALETEGLLLYNGNARGKDFLALALLDGHVQFRFDTGSGPAVLTSLVPVEPGRWHRLELSRHWRQGTLSVDGEAPVVGESPSGTDGLNLDTKLYVGGLPEEQVATVLDRTSVGIGLKGCIRMLDINNQQLELSDWQRAVVQSSGVGECGDHPCSPNPCHGGALCQALEAGVFLCQCPPGRFGPTCADEKNPCQPNPCHGSAPCHVLSRGGAKCACPLGRSGSFCETVLENAGSRPFLADFNGFSYLELKGLHTFERDLGEKMALEMVFLARGPSGLLLYNGQKTDGKGDFVSLALHNRHLEFRYDLGKGAAIIRSKEPIALGTWVRVFLERNGRKGALQVGDGPRVLGESPVPHTMLNLKEPLYVGGAPDFSKLARGAAVASGFDGAIQLVSLRGHQLLTQEHVLRAVDVAPFAGHPCTQAVDNPCLNGGSCIPREATYECLCPGGFSGLHCEKGIVEKSVGDLETLAFDGRTYIEYLNAVTESEKALQSNHFELSLRTEATQGLVLWIGKVGERADYMALAIVDGHLQLSYDLGSQPVVLRSTVKVNTNRWLRVRAHREHREGSLQVGNEAPVTGSSPLGATQLDTDGALWLGGLQKLPVGQALPKAYGTGFVGCLRDVVVGHRQLHLLEDAVTKPELRPCPTL

SEQ ID NO: 10 - DNA, 20 bp, Artificial Sequence
  Single strand DNA oligonucleotide
gtcggctcgcggcaaaaagc

SEQ ID NO: 11 - DNA, 20 bp, Artificial Sequence
  Single strand DNA oligonucleotide
gacatcaaagagaagctgtg

SEQ ID NO: 12 - DNA, 21 bp, Artificial Sequence
  Single strand DNA oligonucleotide
actccataccgataaaggaag

SEQ ID NO: 13 - DNA, 20 bp, Artificial Sequence
  Single strand DNA oligonucleotide
gagagaaagaaaccagagtg

SEQ ID NO: 14 - DNA, 21 bp, Artificial Sequence
  Single strand DNA oligonucleotide
gtctagcaggttcttgaaatc

SEQ ID NO: 15 - DNA, 20 bp, Artificial Sequence
  Single strand DNA oligonucleotide
aattcaagatgcagaagctg

SEQ ID NO: 16 - DNA, 20 bp, Artificial Sequence
  Single strand DNA oligonucleotide
gaattttgaggtctctgctg

SEQ ID NO: 17 - DNA, 21 bp, Artificial Sequence
  Single strand DNA oligonucleotide
ccagaaacatcatcataaccg

SEQ ID NO: 18 - DNA, 20 bp, Artificial Sequence
  Single strand DNA oligonucleotide
catcgccaccttaatagttg

SEQ ID NO: 19 - DNA, 20 bp, Artificial Sequence
  Single strand DNA oligonucleotide
gtcaggctggtcaccttctg

SEQ ID NO: 20 - DNA, 20 bp, Artificial Sequence
  Single strand DNA oligonucleotide
aactcttggcaccatgaacc

SEQ ID NO: 21 - DNA, 22 bp, Artificial Sequence
  Single strand DNA oligonucleotide
gctgggctccctggacattgac

SEQ ID NO: 22 - DNA, 22 bp, Artificial Sequence
  Single strand DNA oligonucleotide
cctgggcctggattctggtgat

SEQ ID NO: 23 - DNA, 25 bp, Artificial Sequence
  Single strand DNA oligonucleotide
ccagtgtgaacttgattttgatgaa

SEQ ID NO: 24 - DNA, 27 bp, Artificial Sequence
  Single strand DNA oligonucleotide
aacataacttgggagacagagacatct

SEQ ID NO: 25 - DNA, 20 bp, Artificial Sequence
  Single strand DNA oligonucleotide
catcgacgcccagatgaaga

SEQ ID NO: 26 - DNA, 20 bp, Artificial Sequence
  Single strand DNA oligonucleotide
tggtgaacagggtcccaaac

SEQ ID NO: 27 - DNA, 18 bp, Artificial Sequence
  Single strand DNA oligonucleotide
cggaggagcgaacacctg

SEQ ID NO: 28 - DNA, 20 bp, Artificial Sequence
  Single strand DNA oligonucleotide
gttggatcctcaccctctgc

SEQ ID NO: 29 - DNA, 20 bp, Artificial Sequence
  Single strand DNA oligonucleotide
ttcgatggtccttgtgaccc

SEQ ID NO: 30 - DNA, 20 bp, Artificial Sequence
  Single strand DNA oligonucleotide
agataggtgtgtgttgggcg

SEQ ID NO: 31 - DNA, 20 bp, Artificial Sequence
  Single strand DNA oligonucleotide
gtgcccatcgtcaacctgaa

SEQ ID NO: 32 - DNA, 20 bp, Artificial Sequence
  Single strand DNA oligonucleotide
agttgaccctgggagccaga

SEQ ID NO: 33 - DNA, 22 bp, Artificial Sequence
  Single strand DNA oligonucleotide
ccttctggcacaagtctcttgg

SEQ ID NO: 34 - DNA, 22 bp, Artificial Sequence
  Single strand DNA oligonucleotide
tcgaagatgacactggcatcgg

SEQ ID NO: 35 - DNA, 20 bp, Artificial Sequence
  Single strand DNA oligonucleotide
tcgagcttgatctctcctat

SEQ ID NO: 36 - DNA, 20 bp, Artificial Sequence
  Single strand DNA oligonucleotide
tggtcccaggtcttacagaa

SEQ ID NO: 37 - DNA, 20 bp, Artificial Sequence
  Single strand DNA oligonucleotide
tggccggcagcgtttctgag

SEQ ID NO: 38 - protein, 4380 aa, Homo sapiens
MGWRAAGALLLALLLHGRLLAVTHGLRAYDGLSLPEDIETVTASQMRWTHSYLSDDEDMLADSISGDDLGSGDLGSGDFQMVYFRALVNFTRSIEYSPQLEDAGSREFREVSEAVVDTLESEYLKIPGDQVVSVVFIKELDGWVFVELDVGSEGNADGAQIQEMLLRVISSGSVASYVTSPQGFQFRRLGTVPQFPRACTEAEFACHSYNECVALEYRCDRRPDCRDMSDELNCEEPVLGISPTFSLLVETTSLPPRPETTIMRQPPVTHAPQPLLPGSVRPLPCGPQEAACRNGHCIPRDYLCDGQEDCEDGSDELDCGPPPPCEPNEFPCGNGHCALKLWRCDGDFDCEDRTDEANCPTKRPEEVCGPTQFRCVSTNMCIPASFHCDEESDCPDRSDEFGCMPPQVVTPPRESIQASRGQTVTFTCVAIGVPTPIINWRLNWGHIPSHPRVTVTSEGGRGTLIIRDVKESDQGAYTCEAMNARGMVFGIPDGVLELVPQRGPCPDGHFYLEHSAACLPCFCFGITSVCQSTRRFRDQIRLRFDQPDDFKGVNVTMPAQPGTPPLSSTQLQIDPSLHEFQLVDLSRRFLVHDSFWALPEQFLGNKVDSYGGSLRYNVRYELARGMLEPVQRPDVVLMGAGYRLLSRGHTPTQPGALNQRQVQFSEEHWVHESGRPVQRAELLQVLQSLEAVLIQTVYNTKMASVGLSDIAMDTTVTHATSHGRAHSVEECRCPIGYSGLSCESCDAHFTRVPGGPYLGTCSGCNCNGHASSCDPVYGHCLNCQHNTEGPQCNKCKAGFFGDAMKATATSCRPCPCPYIDASRRFSDTCFLDTDGQATCDACAPGYTGRRCESCAPGYEGNPIQPGGKCRPVNQEIVRCDERGSMGTSGEACRCKNNVVGRLCNECADGSFHLSTRNPDGCLKCFCMGVSRHCTSSSWSRAQLHGASEEPGHFSLTNAASTHTTNEGIFSPTPGELGFSSFHRLLSGPYFWSLPSRFLGDKVTSYGGELRFTVTQRSQPGSTPLHGQPLVVLQGNNIILEHHVAQEPSPGQPSTFIVPFREQAWQRPDGQPATREHLLMALAGIDTLLIRASYAQQPAESRVSGISMDVAVPEETGQDPALEVEQCSCPPGYRGPSCQDCDTGYTRTPSGLYLGTCERCSCHGHSEACEPETGACQGCQHHTEGPRCEQCQPGYYGDAQRGTPQDCQLCPCYGDPAAGQAAHTCFLDTDGHPTCDACSPGHSGRHCERCAPGYYGNPSQGQPCQRDSQVPGPIGCNCDPQGSVSSQCDAAGQCQCKAQVEGLTCSHCRPHHFHLSASNPDGCLPCFCMGITQQCASSAYTRHLISTHFAPGDFQGFALVNPQRNSRLTGEFTVEPVPEGAQLSFGNFAQLGHESFYWQLPETYQGDKVAAYGGKLRYTLSYTAGPQGSPLSDPDVQITGNNIMLVASQPALQGPERRSYEIMFREEFWRRPDGQPATREHLLMALADLDELLIRATFSSVPLAASISAVSLEVAQPGPSNRPRALEVEECRCPPGYIGLSCQDCAPGYTRTGSGLYLGHCELCECNGHSDLCHPETGACSQCQHNAAGEFCELCAPGYYGDATAGTPEDCQPCACPLTNPENMFSRTCESLGAGGYRCTACEPGYTGQYCEQCGPGYVGNPSVQGGQCLPETNQAPLVVEVHPARSIVPQGGSHSLRCQVSGSPPHYFYWSREDGRPVPSGTQQRHQGSELHFPSVQPSDAGVYICTCRNLHQSNTSRAELLVTEAPSKPITVTVEEQRSQSVRPGADVTFICTAKSKSPAYTLVWTRLHNGKLPTRAMDFNGILTIRNVQLSDAGTYVCTGSNMFAMDQGTATLHVQASGTLSAPVVSIHPPQLTVQPGQLAEFRCSATGSPTPTLEWTGGPGGQLPAKAQIHGGILRLPAVEPTDQAQYLCRAHSSAGQQVARAVLHVHGGGGPRVQVSPERTQVHAGRTVRLYCRAAGVPSATITWRKEGGSLPPQARSERTDIATLLIPAITTADAGFYLCVATSPAGTAQARIQVVVLSASDASPPPVKIESSSPSVTEGQTLDLNCVVAGSAHAQVTWYRRGGSLPPHTQVHGSRLRLPQVSPADSGEYVCRVENGSGPKEASITVSVLHGTHSGPSYTPVPGSTRPIRIEPSSSHVAEGQTLDLNCVVPGQAHAQVTWHKRGGSLPARHQTHGSLLRLHQVTPADSGEYVCHVVGTSGPLEASVLVTIEASVIPGPIPPVRIESSSSTVAEGQTLDLSCVVAGQAHAQVTWYKRGGSLPARHQVRGSRLYIFQASPADAGQYVCRASNGMEASITVTVTGTQGANLAYPAGSTQPIRIEPSSSQVAEGQTLDLNCVVPGQSHAQVTWHKRGGSLPVRHQTHGSLLRLYQASPADSGEYVCRVLGSSVPLEASVLVTIEPAGSVPALGVTPTVRIESSSSQVAEGQTLDLNCLVAGQAHAQVTWHKRGGSLPARHQVHGSRLRLLQVTPADSGEYVCRVVGSSGTQEASVLVTIQQRLSGSHSQGVAYPVRIESSSASLANGHTLDLNCLVASQAPHTITWYKRGGSLPSRHQIVGSRLRIPQVTPADSGEYVCHVSNGAGSRETSLIVTIQGSGSSHVPSVSPPIRIESSSPTVVEGQTLDLNCVVARQPQAIITWYKRGGSLPSRHQTHGSHLRLHQMSVADSGEYVCRANNNIDALEASIVISVSPSAGSPSAPGSSMPIRIESSSSHVAEGETLDLNCVVPGQAHAQVTWHKRGGSLPSHHQTRGSRLRLHHVSPADSGEYVCRVMGSSGPLEASVLVTIEASGSSAVHVPAPGGAPPIRIEPSSSRVAEGQTLDLKCVVPGQAHAQVTWHKRGGNLPARHQVHGPLLRLNQVSPADSGEYSCQVTGSSGTLEASVLVTIEPSSPGPIPAPGLAQPIYIEASSSHVTEGQTLDLNCVVPGQAHAQVTWYKRGGSLPARHQTHGSQLRLHLVSPADSGEYVCRAASGPGPEQEASFTVTVPPSEGSSYRLRSPVISIDPPSSTVQQGQDASFKCLIHDGAAPISLEWKTRNQELEDNVHISPNGSIITIVGTRPSNHGTYRCVASNAYGVAQSVVNLSVHGPPTVSVLPEGPVWVKVGKAVTLECVSAGEPRSSARWTRISSTPAKLEQRTYGLMDSHAVLQISSAKPSDAGTYVCLAQNALGTAQKQVEVIVDTGAMAPGAPQVQAEEAELTVEAGHTATLRCSATGSPAPTIHWSKLRSPLPWQHRLEGDTLIIPRVAQQDSGQYICNATSPAGHAEATIILHVESPPYATTVPEHASVQAGETVQLQCLAHGTPPLTFQWSRVGSSLPGRATARNELLHFERAAPEDSGRYRCRVTNKVGSAEAFAQLLVQGPPGSLPATSIPAGSTPTVQVTPQLETKSIGASVEFHCAVPSDRGTQLRWFKEGGQLPPGHSVQDGVLRIQNLDQSCQGTYICQAHGPWGKAQASAQLVIQALPSVLINIRTSVQTVVVGHAVEFECLALGDPKPQVTWSKVGGHLRPGIVQSGGVVRIAHVELADAGQYRCTATNAAGTTQSHVLLLVQALPQISMPQEVRVPAGSAAVFPCIASGYPTPDISWSKLDGSLPPDSRLENNMLMLPSVRPQDAGTYVCTATNRQGKVKAFAHLQVPERVVPYFTQTPYSFLPLPTIKDAYRKFEIKITFRPDSADGMLLYNGQKRVPGSPTNLANRQPDFISFGLVGGRPEFRFDAGSGMATIRHPTPLALGHFHTVTLLRSLTQGSLIVGDLAPVNGTSQGKFQGLDLNEELYLGGYPDYGAIPKAGLSSGFIGCVRELRIQGEEIVFHDLNLTAHGISHCPTCRDRPCQNGGQCHDSESSSYVCVCPAGFTGSRCEHSQALHCHPEACGPDATCVNRPDGRGYTCRCHLGRSGLRCEEGVTVTTPSLSGAGSYLALPALTNTHHELRLDVEFKPLAPDGVLLFSGGKSGPVEDFVSLAMVGGHLEFRYELGSGLAVLRSAEPLALGRWHRVSAERLNKDGSLRVNGGRPVLRSSPGKSQGLNLHTLLYLGGVEPSVPLSPATNMSAHFRGCVGEVSVNGKRLDLTYSFLGSQGIGQCYDSSPCERQPCQHGATCMPAGEYEFQCLCRDGFKGDLCEHEENPCQLREPCLHGGTCQGTRCLCLPGFSGPRCQQGSGHGIAESDWHLEGSGGNDAPGQYGAYFHDDGFLAFPGHVFSRSLPEVPETIELEVRTSTASGLLLWQGVEVGEAGQGKDFISLGLQDGHLVFRYQLGSGEARLVSEDPINDGEWHRVTALREGRRGSIQVDGEELVSGRSPGPNVAVNAKGSVYIGGAPDVATLTGGRFSSGITGCVKNLVLHSARPGAPPPQPLDLQHRA